European Patent Application EP 4 763 216 A1, published June 24, 2026. Title: Composition for Promoting Hair Growth, or Inhibiting, Preventing or Improving Hair Loss Comprising Peptide As Active Ingredient. Applicant: CAREGEN CO., LTD. The sequence listing filed with the application follows.

SEQUENCE LISTING (47 sequences)

SEQ ID NO: 1 - protein, 5 aa, synthetic construct
GKRRR

SEQ ID NO: 2 - DNA, 20 bp, synthetic construct
  source 1..20: mol_type = other DNA
tgctggtgatgggagttgta

SEQ ID NO: 3 - DNA, 20 bp, synthetic construct
  source 1..20: mol_type = other DNA
cctccaagtagcagccaaag

SEQ ID NO: 4 - DNA, 20 bp, synthetic construct
  source 1..20: mol_type = other DNA
caatgcctctggttcccctt

SEQ ID NO: 5 - DNA, 20 bp, synthetic construct
  source 1..20: mol_type = other DNA
cccctcgaggatttcgacag

SEQ ID NO: 6 - DNA, 22 bp, synthetic construct
  source 1..22: mol_type = other DNA
tctgtcgaacacagtggtacct

SEQ ID NO: 7 - DNA, 23 bp, synthetic construct
  source 1..23: mol_type = other DNA
gtgtgtccatttagctgatgcat

SEQ ID NO: 8 - DNA, 22 bp, synthetic construct
  source 1..22: mol_type = other DNA
atgaactttctgggtcttgggt

SEQ ID NO: 9 - DNA, 22 bp, synthetic construct
  source 1..22: mol_type = other DNA
tggccttggtgaggtttgatcc

SEQ ID NO: 10 - DNA, 20 bp, synthetic construct
  source 1..20: mol_type = other DNA
ggagccaaaagggtcatcat

SEQ ID NO: 11 - DNA, 20 bp, synthetic construct
  source 1..20: mol_type = other DNA
gtgatggcatggactgtggt

SEQ ID NO: 12 - DNA, 20 bp, synthetic construct
  source 1..20: mol_type = other DNA
ccagctattgtaacacctca

SEQ ID NO: 13 - DNA, 20 bp, synthetic construct
  source 1..20: mol_type = other DNA
ttcagatgtaggcagctgtc

SEQ ID NO: 14 - DNA, 28 bp, synthetic construct
  source 1..28: mol_type = other DNA
accttcgttgccctctgtgccacagatg

SEQ ID NO: 15 - DNA, 21 bp, synthetic construct
  source 1..21: mol_type = other DNA
aggcccggaggcagtccgggt

SEQ ID NO: 16 - DNA, 25 bp, synthetic construct
  source 1..25: mol_type = other DNA
accagcagcgactctgaggaggaac

SEQ ID NO: 17 - DNA, 26 bp, synthetic construct
  source 1..26: mol_type = other DNA
tgaccctcttggcagcaggatagtcc

SEQ ID NO: 18 - DNA, 20 bp, synthetic construct
  source 1..20: mol_type = other DNA
gatcatcgagctgagacgca

SEQ ID NO: 19 - DNA, 20 bp, synthetic construct
  source 1..20: mol_type = other DNA
ctggccccagggtatctagt

SEQ ID NO: 20 - DNA, 20 bp, synthetic construct
  source 1..20: mol_type = other DNA
cgcggcgtatccgtgtcctc

SEQ ID NO: 21 - DNA, 24 bp, synthetic construct
  source 1..24: mol_type = other DNA
agcctgttccgtctcaaacttggt

SEQ ID NO: 22 - DNA, 20 bp, synthetic construct
  source 1..20: mol_type = other DNA
ccaaatccgcaccaaggtca

SEQ ID NO: 23 - DNA, 21 bp, synthetic construct
  source 1..21: mol_type = other DNA
gtattgattgccaggaggggg

SEQ ID NO: 24 - DNA, 20 bp, synthetic construct
  source 1..20: mol_type = other DNA
ccctcaaggatgccaggaac

SEQ ID NO: 25 - DNA, 19 bp, synthetic construct
  source 1..19: mol_type = other DNA
cactgctacctccggcaag

SEQ ID NO: 26 - DNA, 20 bp, synthetic construct
  source 1..20: mol_type = other DNA
cggtcaagtcggaaaattca

SEQ ID NO: 27 - DNA, 20 bp, synthetic construct
  source 1..20: mol_type = other DNA
gaggagctgggatgtggtaa

SEQ ID NO: 28 - DNA, 20 bp, synthetic construct
  source 1..20: mol_type = other DNA
gccgtctatacggacatgcc

SEQ ID NO: 29 - DNA, 20 bp, synthetic construct
  source 1..20: mol_type = other DNA
gcagtacacctgactgtccc

SEQ ID NO: 30 - DNA, 20 bp, synthetic construct
  source 1..20: mol_type = other DNA
caggactgggtgatggtgtc

SEQ ID NO: 31 - DNA, 20 bp, synthetic construct
  source 1..20: mol_type = other DNA
tctgagggtgagagcctgaa

SEQ ID NO: 32 - DNA, 20 bp, synthetic construct
  source 1..20: mol_type = other DNA
ctgcatgcaagagtgacacc

SEQ ID NO: 33 - DNA, 20 bp, synthetic construct
  source 1..20: mol_type = other DNA
gacattgccccttccctttg

SEQ ID NO: 34 - DNA, 19 bp, synthetic construct
  source 1..19: mol_type = other DNA
gagaccaaagaggcgttgg

SEQ ID NO: 35 - DNA, 20 bp, synthetic construct
  source 1..20: mol_type = other DNA
ggctagttttcacgctggtc

SEQ ID NO: 36 - DNA, 20 bp, synthetic construct
  source 1..20: mol_type = other DNA
ccagcaagacggagatcaca

SEQ ID NO: 37 - DNA, 20 bp, synthetic construct
  source 1..20: mol_type = other DNA
gaagaggcttccctgatggc

SEQ ID NO: 38 - DNA, 20 bp, synthetic construct
  source 1..20: mol_type = other DNA
aagctgcaacgaaaacgacg

SEQ ID NO: 39 - DNA, 20 bp, synthetic construct
  source 1..20: mol_type = other DNA
ggtggggctagtcaagtctg

SEQ ID NO: 40 - DNA, 20 bp, synthetic construct
  source 1..20: mol_type = other DNA
cctatccccgggactaagac

SEQ ID NO: 41 - DNA, 20 bp, synthetic construct
  source 1..20: mol_type = other DNA
atgctcttcaggggcaacac

SEQ ID NO: 42 - DNA, 20 bp, synthetic construct
  source 1..20: mol_type = other DNA
tggaccagctaaccaacgac

SEQ ID NO: 43 - DNA, 20 bp, synthetic construct
  source 1..20: mol_type = other DNA
gtcattgttccggttggcag

SEQ ID NO: 44 - DNA, 20 bp, synthetic construct
  source 1..20: mol_type = other DNA
gcctgggaggttctggattc

SEQ ID NO: 45 - DNA, 20 bp, synthetic construct
  source 1..20: mol_type = other DNA
ggagagagcaggctttggtt

SEQ ID NO: 46 - DNA, 20 bp, synthetic construct
  source 1..20: mol_type = other DNA
cccagccaacctatgaggag

SEQ ID NO: 47 - DNA, 20 bp, synthetic construct
  source 1..20: mol_type = other DNA
cttgaggagaccagcaccac